European Patent Application EP 4 421 087 A1, published August 28, 2024. Title: STAPLE-CONTAINING POLYPEPTIDES AND APPLICATION THEREOF. Applicant: MEDSHINE DISCOVERY INC. Application WO. The sequence listing filed with the application follows.

SEQUENCE LISTING (5 sequences)

SEQ ID NO: 1 - protein, 34 aa, synthetic construct
  MOD_RES 17: note = 1Lys
  MOD_RES 20: note = 1Lys
  VARIANT 2: note = Aib
  VARIANT 34: note = X2
HXQGTFTSDYSKYLDEKKAKEFVEWLLEGGPSSX

SEQ ID NO: 2 - protein, 34 aa, synthetic construct
  VARIANT 2: note = Aib
  VARIANT 34: note = X2
  MOD_RES 17: note = 1Lys
  MOD_RES 21: note = 1Lys
HXQGTFTSDYSKYLDEKKAKKFVEWLLEGGPSSX

SEQ ID NO: 3 - protein, 34 aa, synthetic construct; identical to SEQ ID NO: 2
  VARIANT 2: note = Aib
  VARIANT 34: note = X2
  MOD_RES 18: note = 1Lys
  MOD_RES 21: note = 1Lys

SEQ ID NO: 4 - protein, 34 aa, synthetic construct
  VARIANT 2: note = Aib
  VARIANT 34: note = X2
  MOD_RES 20: note = 1Lys
  MOD_RES 24: note = 1Lys
HXQGTFTSDYSKYLDEKKAKEFVKWLLEGGPSSX

SEQ ID NO: 5 - protein, 34 aa, synthetic construct
  VARIANT 2: note = Aib
  VARIANT 34: note = X2
  MOD_RES 24: note = 1Lys
  MOD_RES 28: note = 1Lys
HXQGTFTSDYSKYLDEKKAKEFVKWLLKGGPSSX